European Patent Specification EP 3 277 316 B1, published March 5, 2025. Title: Bispecific CXCR4-CD4 Polypeptides with potent anti-HIV activity. Applicant: Ablynx N.V. The sequence listing filed with the application follows.

SEQUENCE LISTING (136 sequences)

SEQ ID NO: 1 - protein, 458 aa, Homo sapiens
MNRGVPFRHLLLVLQLALLPAATQGKKVVLGKKGDTVELTCTASQKKSIQFHWKNSNQIKILGNQGSFLTKGPSKLNDRADSRRSLWDQGNFPLIIKNLKIEDSDTYICEVEDQKEEVQLLVFGLTANSDTHLLQGQSLTLTLESPPGSSPSVQCRSPRGKNIQGGKTLSVSQLELQDSGTWTCTVLQNQKKVEFKIDIVVLAFQKASSIVYKKEGEQVEFSFPLAFTVEKLTGSGELWWQAERASSSKSWITFDLKNKEVSVKRVTQDPKLQMGKKLPLHLTLPQALPQYAGSGNLTLALEAKTGKLHQEVNLVVMRATQLQKNLTCEVWGPTSPKLMLSLKLENKEAKVSKREKAVWVLNPEAGMWQCLLSDSGQVLLESNIKVLPTWSTPVQPMALIVLGGVAGLLLFIGLGIFFCVRCRHRRRQAERMSQIKRLLSEKKTCQCPHRFQKTCSPI

SEQ ID NO: 2 - protein, 360 aa, Homo sapiens [sequence omitted]

SEQ ID NO: 3 - protein, 352 aa, Homo sapiens [sequence omitted]

SEQ ID NO: 4 - protein, 128 aa, Artificial Sequence
  Nanobody Sequence
EVQLMESGGGLVQAGGSLRLSCAASGRTFNNYAMGWFRRAPGKEREFVAAITRSGVRSGVSAIYGDSVKDRFTISRDNAKNTLYLQMNSLKPEDTAVYTCAASAIGSGALRRFEYDYSGQGTQVTVSS

SEQ ID NO: 5 - protein, 128 aa, Artificial Sequence
  Nanobody Sequence
EVQLVESGGGLVQAGGSLRLSCAASGRTFNNYAMGWFRRAPGKEREFVAAITRSGVRSGVSAIYGDSVKDRFTISRDNAKNTLYLQMNSLKPEDTAVYTCAASAIGSGALRRFEYDYSGQGTQVTVSS

SEQ ID NO: 6 - protein, 128 aa, Artificial Sequence
  Nanobody Sequence
EVQLVESGGGLVQAGGSLRLSCKASGGTFNNYAMGWFRRAPGKEREFVAAITRSGVRSGVSAIYGDSVKDRFTISRDNVKNTLYLQMNTLKPEDTAVYTCAASAIGSGALRRFEYDYSGQGTQVTVSS

SEQ ID NO: 7 - protein, 128 aa, Artificial Sequence
  Nanobody Sequence
EVQLVESGGGLVQAGGSLRLSCAASGGTFNNYAMGWFRRAPGKEREFVAAISRSGVRTGVSALYGDSVKDRFTISRDNAKNTLYLQMNKMKPEDTAVYTCAASAIGSGALRRFEYDSSGQGTQVTVSS

SEQ ID NO: 8 - protein, 128 aa, Artificial Sequence
  Nanobody Sequence
EVQLVESGGGLVQTGGSLRLSCAASGGTFNNYAMGWFRRAPGKEREFVAAISRSGVRTGVSALYGDSVKDRFTISRDNAKNTLYLQMNKMKPEDTAVYTCAASAIGSGALRRFEYDSSGQGTQVTVSS

SEQ ID NO: 9 - protein, 126 aa, Artificial Sequence
  Nanobody Sequence
EVQLVESGGGLVQAGDSLRLSCAASGRAFSRYAMGWFRQAPGKEREFVAAIGWGPSKTNYADSVKGRFTISRDNAKNTVYLQMNTLKPEDTAVYSCAAKFVNTDSTWSRSEMYTYWGQGTQVTVSS

SEQ ID NO: 10 - protein, 119 aa, Artificial Sequence
  Nanobody Sequence
EVQLVASGGGLVQAGGSLRLSCAVSGTTFSVATLGWYRQAPGQQRALVADISSGGSTNYADSVRGRFTISRDNAKNLAYLQMNSLKPEDTAVYYCNARTSGWRTRSNYWGQGTQVTVSS

SEQ ID NO: 11 - protein, 119 aa, Artificial Sequence
  Nanobody Sequence
EVQLVESGGGLVQAGGSLRLSCAVSGTTFSVATLGWYRQAPGQQRALVADISSGGSTNYADSVRGRFTISRDNAKNLAYLQMNSLKPEDTAVYYCNARTSGWRTRSNYWGQGTQVTVSS

SEQ ID NO: 12 - protein, 122 aa, Artificial Sequence
  Nanobody Sequence
EVQLVESGGGLVQAGGSLRLSCVASVNIFGSIAMAWYRQAPGKQRNLVASISSGGRINYADSRKGRFTISRDNTKNTVHLQMNSLEPEDTAVYYCAAGRIGQRTLTFTPDYWGQGTQVTVSS

SEQ ID NO: 13 - protein, 126 aa, Artificial Sequence
  Nanobody Sequence
EVQLVESGGGLVRAGDSLRLSCAASGRAFSRYAMGWFRQALGKERELVAAIGWSPTHTYYADSVKGRFTMSRDNGKNTVFLQMNSLNPEDTAVYYCAAKYSSRDAAYRSDYDYNYWGQGTQVTVSS

SEQ ID NO: 14 - protein, 128 aa, Artificial Sequence
  Nanobody Sequence
EVQLVESGGGLVQAGDSLRVSCAASGRTSSYAMAWFRQAPGKEREFVGTISRTNSRTKYADFVEGRFTISRDNAKSTLSLQMTSLKPEDTAVYYCAAKWTGNSYHDYTWSKVDEYNVWGQGTQVTVSS

SEQ ID NO: 15 - protein, 121 aa, Artificial Sequence
  Nanobody Sequence
EVQLVESGGGLVQAGGSLRLSCAASGRTFSRAAMGWFRQAPGKEREFVGCALSSAGSALTADSVKGRFTISRDNAKNMVYLQMNNLKPEDTAVYSCVAGGYCTRAGVYPYWGQGTQVTVSS

SEQ ID NO: 16 - protein, 120 aa, Artificial Sequence
  Nanobody Sequence
EVQLVESGGGLVQPGGSLRLSCAASGTIFSTSTMGWYSQAPGKQRELVADITFLGSAKYADSVKGRFTISRDKIKNTVYLQMNSLKPEDTAAYYCNARQSTFRGVHYNYWGQGTQVTVSS

SEQ ID NO: 17 - protein, 121 aa, Artificial Sequence
  Nanobody Sequence
EVQLVESGGGLVQSGGSLRLSCAASGFTFSGYWMYWVRQAPGKGLEWVSAISPGGGSTYYPDSVKGRFTISRDNAKNTLYLQMNSLKPEDTALYYCASSLTATHTYEYDYWGQGTQVTVSS

SEQ ID NO: 18 - protein, 122 aa, Artificial Sequence
  Nanobody Sequence
EVQLVESGGGLVQAGGSLRLSCAASGRTSASYSMGWFRQAPGKEREFVAAISWSGDETSYADSVKGRFTIARGNAKNTVYLQMNSLKSEDTAIYYCAGDRWWRPAGLQWDYWGQGTQVTVSS

SEQ ID NO: 19 - protein, 117 aa, Artificial Sequence
  Nanobody Sequence
EVQLVESGGGLVQAGGSLKLSCAASRSILDFNAMGWYRQAPGKQREWVTTIARAGATKYADSVKGRFSISRDNAKNTVYLQMSSLKPEDTATYYCNARVFDLPNDYWGQGTQVTVSS

SEQ ID NO: 20 - protein, 125 aa, Artificial Sequence
  Nanobody Sequence
EVQLVESGGGSVQPGGSLTLSCGTSGRTFNVMGWFRQAPGKEREFVAAVRWSSTGIYYTQYADSVKSRFTISRDNAKNTVYLEMNSLKPEDTAVYYCAADTYNSNPARWDGYDFRGQGTQVTVSS

SEQ ID NO: 21 - protein, 30 aa, Artificial Sequence
  Framework 1
EVQLMESGGGLVQAGGSLRLSCAASGRTFN

SEQ ID NO: 22 - protein, 30 aa, Artificial Sequence
  Framework 1
EVQLVESGGGLVQAGGSLRLSCAASGRTFN

SEQ ID NO: 23 - protein, 30 aa, Artificial Sequence
  Framework 1
EVQLVESGGGLVQAGGSLRLSCKASGGTFN

SEQ ID NO: 24 - protein, 30 aa, Artificial Sequence
  Framework 1
EVQLVESGGGLVQAGGSLRLSCAASGGTFN

SEQ ID NO: 25 - protein, 30 aa, Artificial Sequence
  Framework 1
EVQLVESGGGLVQTGGSLRLSCAASGGTFN

SEQ ID NO: 26 - protein, 30 aa, Artificial Sequence
  Framework 1
EVQLVESGGGLVQAGDSLRLSCAASGRAFS

SEQ ID NO: 27 - protein, 30 aa, Artificial Sequence
  Framework 1
EVQLVASGGGLVQAGGSLRLSCAVSGTTFS

SEQ ID NO: 28 - protein, 30 aa, Artificial Sequence
  Framework 1
EVQLVESGGGLVQAGGSLRLSCAVSGTTFS

SEQ ID NO: 29 - protein, 30 aa, Artificial Sequence
  Framework 1
EVQLVESGGGLVQAGGSLRLSCVASVNIFG

SEQ ID NO: 30 - protein, 30 aa, Artificial Sequence
  Framework 1
EVQLVESGGGLVRAGDSLRLSCAASGRAFS

SEQ ID NO: 31 - protein, 29 aa, Artificial Sequence
  Framework 1
EVQLVESGGGLVQAGDSLRVSCAASGRTS

SEQ ID NO: 32 - protein, 29 aa, Artificial Sequence
  Framework 1
EVQLVESGGGLVQAGGSLRLSCAASGRTF

SEQ ID NO: 33 - protein, 29 aa, Artificial Sequence
  Framework 1
EVQLVESGGGLVQPGGSLRLSCAASGTIF

SEQ ID NO: 34 - protein, 5 aa, Artificial Sequence
  CDR1
NYAMG

SEQ ID NO: 35 - protein, 5 aa, Artificial Sequence
  CDR1
RYAMG

SEQ ID NO: 36 - protein, 5 aa, Artificial Sequence
  CDR1
VATLG

SEQ ID NO: 37 - protein, 5 aa, Artificial Sequence
  CDR1
SIAMA

SEQ ID NO: 38 - protein, 5 aa, Artificial Sequence
  CDR1
SYAMA

SEQ ID NO: 39 - protein, 6 aa, Artificial Sequence
  CDR1
SRAAMG

SEQ ID NO: 40 - protein, 6 aa, Artificial Sequence
  CDR1
STSTMG

SEQ ID NO: 41 - protein, 14 aa, Artificial Sequence
  Framework 2
WFRRAPGKEREFVA

SEQ ID NO: 42 - protein, 14 aa, Artificial Sequence
  Framework 2
WFRQAPGKEREFVA

SEQ ID NO: 43 - protein, 14 aa, Artificial Sequence
  Framework 2
WYRQAPGQQRALVA

SEQ ID NO: 44 - protein, 14 aa, Artificial Sequence
  Framework 2
WYRQAPGKQRNLVA

SEQ ID NO: 45 - protein, 14 aa, Artificial Sequence
  Framework 2
WFRQALGKERELVA

SEQ ID NO: 46 - protein, 14 aa, Artificial Sequence
  Framework 2
WFRQAPGKEREFVG

SEQ ID NO: 47 - protein, 14 aa, Artificial Sequence
  Framework 2
WYSQAPGKQRELVA

SEQ ID NO: 48 - protein, 21 aa, Artificial Sequence
  CDR 2
AITRSGVRSGVSAIYGDSVKD

SEQ ID NO: 49 - protein, 21 aa, Artificial Sequence
  CDR 2
AISRSGVRTGVSALYGDSVKD

SEQ ID NO: 50 - protein, 17 aa, Artificial Sequence
  CDR 2
AIGWGPSKTNYADSVKG

SEQ ID NO: 51 - protein, 16 aa, Artificial Sequence
  CDR 2
DISSGGSTNYADSVRG

SEQ ID NO: 52 - protein, 16 aa, Artificial Sequence
  CDR 2
SISSGGRINYADSRKG

SEQ ID NO: 53 - protein, 17 aa, Artificial Sequence
  CDR 2
AIGWSPTHTYYADSVKG

SEQ ID NO: 54 - protein, 17 aa, Artificial Sequence
  CDR 2
TISRTNSRTKYADFVEG

SEQ ID NO: 55 - protein, 17 aa, Artificial Sequence
  CDR 2
CALSSAGSALTADSVKG

SEQ ID NO: 56 - protein, 16 aa, Artificial Sequence
  CDR 2
DITFLGSAKYADSVKG

SEQ ID NO: 57 - protein, 32 aa, Artificial Sequence
  Framework 3
RFTISRDNAKNTLYLQMNSLKPEDTAVYTCAA

SEQ ID NO: 58 - protein, 32 aa, Artificial Sequence
  Framework 3
RFTISRDNVKNTLYLQMNTLKPEDTAVYTCAA

SEQ ID NO: 59 - protein, 32 aa, Artificial Sequence
  Framework 3
RFTISRDNAKNTLYLQMNKMKPEDTAVYTCAA

SEQ ID NO: 60 - protein, 32 aa, Artificial Sequence
  Framework 3
RFTISRDNAKNTVYLQMNTLKPEDTAVYSCAA

SEQ ID NO: 61 - protein, 32 aa, Artificial Sequence
  Framework 3
RFTISRDNAKNLAYLQMNSLKPEDTAVYYCNA

SEQ ID NO: 62 - protein, 32 aa, Artificial Sequence
  Framework 3
RFTISRDNTKNTVHLQMNSLEPEDTAVYYCAA

SEQ ID NO: 63 - protein, 32 aa, Artificial Sequence
  Framework 3
RFTMSRDNGKNTVFLQMNSLNPEDTAVYYCAA

SEQ ID NO: 64 - protein, 32 aa, Artificial Sequence
  Framework 3
RFTISRDNAKSTLSLQMTSLKPEDTAVYYCAA

SEQ ID NO: 65 - protein, 32 aa, Artificial Sequence
  Framework 3
RFTISRDNAKNMVYLQMNNLKPEDTAVYSCVA

SEQ ID NO: 66 - protein, 32 aa, Artificial Sequence
  Framework 3
RFTISRDKIKNTVYLQMNSLKPEDTAAYYCNA

SEQ ID NO: 67 - protein, 15 aa, Artificial Sequence
  CDR 3
SAIGSGALRRFEYDY

SEQ ID NO: 68 - protein, 15 aa, Artificial Sequence
  CDR 3
SAIGSGALRRFEYDS

SEQ ID NO: 69 - protein, 17 aa, Artificial Sequence
  CDR 3
KFVNTDSTWSRSEMYTY

SEQ ID NO: 70 - protein, 11 aa, Artificial Sequence
  CDR 3
RTSGWRTRSNY

SEQ ID NO: 71 - protein, 14 aa, Artificial Sequence
  CDR 3
GRIGQRTLTFTPDY

SEQ ID NO: 72 - protein, 17 aa, Artificial Sequence
  CDR 3
KYSSRDAAYRSDYDYNY

SEQ ID NO: 73 - protein, 20 aa, Artificial Sequence
  CDR 3
KWTGNSYHDYTWSKVDEYNV

SEQ ID NO: 74 - protein, 12 aa, Artificial Sequence
  CDR 3
GGYCTRAGVYPY

SEQ ID NO: 75 - protein, 12 aa, Artificial Sequence
  CDR 3
RQSTFRGVHYNY

SEQ ID NO: 76 - protein, 11 aa, Artificial Sequence
  Framework 4
SGQGTQVTVSS

SEQ ID NO: 77 - protein, 11 aa, Artificial Sequence
  Framework 4
WGQGTQVTVSS

SEQ ID NO: 78 - protein, 30 aa, Artificial Sequence
  Framework 1
EVQLVESGGGLVQSGGSLRLSCAASGFTFS

SEQ ID NO: 79 - protein, 30 aa, Artificial Sequence
  Framework 1
EVQLVESGGGLVQAGGSLRLSCAASGRTSA

SEQ ID NO: 80 - protein, 30 aa, Artificial Sequence
  Framework 1
EVQLVESGGGLVQAGGSLKLSCAASRSILD

SEQ ID NO: 81 - protein, 30 aa, Artificial Sequence
  Framework 1
EVQLVESGGGSVQPGGSLTLSCGTSGRTFN

SEQ ID NO: 82 - protein, 5 aa, Artificial Sequence
  CDR 1
GYWMY

SEQ ID NO: 83 - protein, 5 aa, Artificial Sequence
  CDR 1
SYSMG

SEQ ID NO: 84 - protein, 5 aa, Artificial Sequence
  CDR 1
FNAMG

SEQ ID NO: 85 - protein, 3 aa, Artificial Sequence
  CDR 1
VMG

SEQ ID NO: 86 - protein, 14 aa, Artificial Sequence
  Framework 2
WVRQAPGKGLEWVS

SEQ ID NO: 87 - protein, 14 aa, Artificial Sequence
  Framework 2
WYRQAPGKQREWVT

SEQ ID NO: 88 - protein, 17 aa, Artificial Sequence
  CDR 2
AISPGGGSTYYPDSVKG

SEQ ID NO: 89 - protein, 17 aa, Artificial Sequence
  CDR 2
AISWSGDETSYADSVKG

SEQ ID NO: 90 - protein, 16 aa, Artificial Sequence
  CDR 2
TIARAGATKYADSVKG

SEQ ID NO: 91 - protein, 20 aa, Artificial Sequence
  CDR 2
AVRWSSTGIYYTQYADSVKS

SEQ ID NO: 92 - protein, 32 aa, Artificial Sequence
  Framework 3
RFTISRDNAKNTLYLQMNSLKPEDTALYYCAS

SEQ ID NO: 93 - protein, 32 aa, Artificial Sequence
  Framework 3
RFTIARGNAKNTVYLQMNSLKSEDTAIYYCAG

SEQ ID NO: 94 - protein, 32 aa, Artificial Sequence
  Framework 3
RFSISRDNAKNTVYLQMSSLKPEDTATYYCNA

SEQ ID NO: 95 - protein, 32 aa, Artificial Sequence
  Framework 3
RFTISRDNAKNTVYLEMNSLKPEDTAVYYCAA

SEQ ID NO: 96 - protein, 12 aa, Artificial Sequence
  CDR 3
SLTATHTYEYDY

SEQ ID NO: 97 - protein, 13 aa, Artificial Sequence
  CDR 3
DRWWRPAGLQWDY

SEQ ID NO: 98 - protein, 9 aa, Artificial Sequence
  CDR 3
RVFDLPNDY

SEQ ID NO: 99 - protein, 15 aa, Artificial Sequence
  CDR 3
DTYNSNPARWDGYDF

SEQ ID NO: 100 - protein, 11 aa, Artificial Sequence
  Framework 4
RGQGTQVTVSS

SEQ ID NO: 101 - protein, 261 aa, Artificial Sequence
  Nanobody Sequence
EVQLVESGGGSVQPGGSLTLSCGTSGRTFNVMGWFRQAPGKEREFVAAVRWSSTGIYYTQYADSVKSRFTISRDNAKNTVYLEMNSLKPEDTAVYYCAADTYNSNPARWDGYDFRGQGTQVTVSSGGGGSGGGGSEVQLVESGGGLVQAGDSLRLSCAASGRAFSRYAMGWFRQAPGKEREFVAAIGWGPSKTNYADSVKGRFTISRDNAKNTVYLQMNTLKPEDTAVYSCAAKFVNTDSTWSRSEMYTYWGQGTQVTVSS

SEQ ID NO: 102 - protein, 276 aa, Artificial Sequence
  Nanobody Sequence
EVQLVESGGGSVQPGGSLTLSCGTSGRTFNVMGWFRQAPGKEREFVAAVRWSSTGIYYTQYADSVKSRFTISRDNAKNTVYLEMNSLKPEDTAVYYCAADTYNSNPARWDGYDFRGQGTQVTVSSGGGGSGGGGSGGGGSGGGGSGGGGSEVQLVESGGGLVQAGDSLRLSCAASGRAFSRYAMGWFRQAPGKEREFVAAIGWGPSKTNYADSVKGRFTISRDNAKNTVYLQMNTLKPEDTAVYSCAAKFVNTDSTWSRSEMYTYWGQGTQVTVSS

SEQ ID NO: 103 - protein, 286 aa, Artificial Sequence
  Nanobody Sequence
EVQLVESGGGSVQPGGSLTLSCGTSGRTFNVMGWFRQAPGKEREFVAAVRWSSTGIYYTQYADSVKSRFTISRDNAKNTVYLEMNSLKPEDTAVYYCAADTYNSNPARWDGYDFRGQGTQVTVSSGGGGSGGGGSGGGGSGGGGSGGGGSGGGGSGGGGSEVQLVESGGGLVQAGDSLRLSCAASGRAFSRYAMGWFRQAPGKEREFVAAIGWGPSKTNYADSVKGRFTISRDNAKNTVYLQMNTLKPEDTAVYSCAAKFVNTDSTWSRSEMYTYWGQGTQVTVSS

SEQ ID NO: 104 - protein, 260 aa, Artificial Sequence
  Nanobody Sequence
EVQLVESGGGLVQAGDSLRLSCAASGRAFSRYAMGWFRQAPGKEREFVAAIGWGPSKTNYADSVKGRFTISRDNAKNTVYLQMNTLKPEDTAVYSCAAKFVNTDSTWSRSEMYTYWGQGTQVTVSSGGGSGGGGSEVQLVESGGGSVQPGGSLTLSCGTSGRTFNVMGWFRQAPGKEREFVAAVRWSSTGIYYTQYADSVKSRFTISRDNAKNTVYLEMNSLKPEDTAVYYCAADTYNSNPARWDGYDFRGQGTQVTVSS

SEQ ID NO: 105 - protein, 276 aa, Artificial Sequence
  Nanobody Sequence
EVQLVESGGGLVQAGDSLRLSCAASGRAFSRYAMGWFRQAPGKEREFVAAIGWGPSKTNYADSVKGRFTISRDNAKNTVYLQMNTLKPEDTAVYSCAAKFVNTDSTWSRSEMYTYWGQGTQVTVSSGGGGSGGGGSGGGGSGGGGSGGGGSEVQLVESGGGSVQPGGSLTLSCGTSGRTFNVMGWFRQAPGKEREFVAAVRWSSTGIYYTQYADSVKSRFTISRDNAKNTVYLEMNSLKPEDTAVYYCAADTYNSNPARWDGYDFRGQGTQVTVSS

SEQ ID NO: 106 - protein, 286 aa, Artificial Sequence
  Nanobody Sequence
EVQLVESGGGLVQAGDSLRLSCAASGRAFSRYAMGWFRQAPGKEREFVAAIGWGPSKTNYADSVKGRFTISRDNAKNTVYLQMNTLKPEDTAVYSCAAKFVNTDSTWSRSEMYTYWGQGTQVTVSSGGGGSGGGGSGGGGSGGGGSGGGGSGGGGSGGGGSEVQLVESGGGSVQPGGSLTLSCGTSGRTFNVMGWFRQAPGKEREFVAAVRWSSTGIYYTQYADSVKSRFTISRDNAKNTVYLEMNSLKPEDTAVYYCAADTYNSNPARWDGYDFRGQGTQVTVSS

SEQ ID NO: 107 - protein, 398 aa, Artificial Sequence
  Nanobody Sequence
EVQLVESGGGLVQAGDSLRVSCAASGRTSSYAMAWFRQAPGKEREFVGTISRTNSRTKYADFVEGRFTISRDNAKSTLSLQMTSLKPEDTAVYYCAAKWTGNSYHDYTWSKVDEYNVWGQGTLVTVSSGGGGSGGGGSGGGGSEVQLVESGGGLVQPGNSLRLSCAASGFTFSSFGMSWVRQAPGKGLEWVSSISGSGSDTLYADSVKGRFTISRDNAKTTLYLQMNSLRPEDTAVYYCTIGGSLSRSSQGTLVTVSSGGGGSGGGGSGGGGSEVQLVESGGGSVQPGGSLTLSCGTSGRTFNVMGWFRQAPGKEREFVAAVRWSSTGIYYTQYADSVKSRFTISRDNAKNTVYLEMNSLKPEDTAVYYCAADTYNSNPARWDGYDFRGQGTLVTVSS

SEQ ID NO: 108 - protein, 396 aa, Artificial Sequence
  Nanobody Sequence
EVQLVESGGGLVRAGDSLRLSCAASGRAFSRYAMGWFRQALGKERELVAAIGWSPTHTYYADSVKGRFTMSRDNGKNTVFLQMNSLNPEDTAVYYCAAKYSSRDAAYRSDYDYNYWGQGTLVTVSSGGGGSGGGGSGGGGSEVQLVESGGGLVQPGNSLRLSCAASGFTFSSFGMSWVRQAPGKGLEWVSSISGSGSDTLYADSVKGRFTISRDNAKTTLYLQMNSLRPEDTAVYYCTIGGSLSRSSQGTLVTVSSGGGGSGGGGSGGGGSEVQLVESGGGSVQPGGSLTLSCGTSGRTFNVMGWFRQAPGKEREFVAAVRWSSTGIYYTQYADSVKSRFTISRDNAKNTVYLEMNSLKPEDTAVYYCAADTYNSNPARWDGYDFRGQGTLVTVSS

SEQ ID NO: 109 - protein, 396 aa, Artificial Sequence
  Nanobody Sequence
EVQLVESGGGLVQAGDSLRLSCAASGRAFSRYAMGWFRQAPGKEREFVAAIGWGPSKTNYADSVKGRFTISRDNAKNTVYLQMNTLKPEDTAVYSCAAKFVNTDSTWSRSEMYTYWGQGTLVTVSSGGGGSGGGGSGGGGSEVQLVESGGGLVQPGNSLRLSCAASGFTFSSFGMSWVRQAPGKGLEWVSSISGSGSDTLYADSVKGRFTISRDNAKTTLYLQMNSLRPEDTAVYYCTIGGSLSRSSQGTLVTVSSGGGGSGGGGSGGGGSEVQLVESGGGSVQPGGSLTLSCGTSGRTFNVMGWFRQAPGKEREFVAAVRWSSTGIYYTQYADSVKSRFTISRDNAKNTVYLEMNSLKPEDTAVYYCAADTYNSNPARWDGYDFRGQGTLVTVSS

SEQ ID NO: 110 - protein, 256 aa, Artificial Sequence
  Nanobody Sequence
EVQLVESGGGLVQAGDSLRLSCAASGRAFSRYAMGWFRQAPGKEREFVAAIGWGPSKTNYADSVKGRFTISRDNAKNTVYLQMNTLKPEDTAVYSCAAKFVNTDSTWSRSEMYTYWGQGTLVTVSSGGGGSGGGGSGGGGSEVQLVESGGGLVQPGNSLRLSCAASGFTFSSFGMSWVRQAPGKGLEWVSSISGSGSDTLYADSVKGRFTISRDNAKTTLYLQMNSLRPEDTAVYYCTIGGSLSRSSQGTLVTVSS

SEQ ID NO: 111 - protein, 115 aa, Artificial Sequence [sequence omitted]

SEQ ID NO: 112 - protein, 115 aa, Artificial Sequence [sequence omitted]

SEQ ID NO: 113 - protein, 116 aa, Artificial Sequence
  Nanobody Sequence
EVQLVESGGGVVQPGNSLRLSCAASGFTFSSFGMSWVRQAPGKGLEWVSSISGSGSDTLYADSVKGRFTISRDNAKTTLYLQMNSLRPEDTATYYCTIGGSLSRSSQGTLVTVSSA

SEQ ID NO: 114 - protein, 116 aa, Artificial Sequence
  Nanobody Sequence
EVQLVESGGGVVQPGGSLRLSCAASGFTFRSFGMSWVRQAPGKGPEWVSSISGSGSDTLYADSVKGRFTISRDNSKNTLYLQMNSLRPEDTATYYCTIGGSLSRSSQGTLVTVSSA

SEQ ID NO: 115 - protein, 115 aa, Artificial Sequence [sequence omitted]

SEQ ID NO: 116 - protein, 116 aa, Artificial Sequence
  Nanobody Sequence
EVQLVESGGGLVQPGNSLRLSCAASGFTFSSFGMSWVRQAPGKGLEWVSSISGSGSDTLYADSVKGRFTISRDNAKTTLYLQMNSLRPEDTAVYYCTIGGSLSRSSQGTLVKVSSA

SEQ ID NO: 117 - protein, 115 aa, Artificial Sequence
  Nanobody Sequence
EVQLVESGGGVVQPGNSLRLSCAASGFTFSSFGMSWVRQAPGKGLEWVSSISGSGSDTLYADSVKGRFTISRDNAKTTLYLQMNSLRPEDTALYYCTIGGSLSRSSQGTLVTVSS

SEQ ID NO: 118 - protein, 116 aa, Artificial Sequence
  Nanobody Sequence
EVQLVESGGGVVQPGNSLRLSCAASGFTFSSFGMSWVRQAPGKGLEWVSSISGSGSDTLYADSVKGRFTISRDNAKTTLYLQMNSLRPEDTALYYCTIGGSLSRSSQGTLVTVSSA

SEQ ID NO: 119 - protein, 117 aa, Artificial Sequence
  Nanobody Sequence
EVQLVESGGGVVQPGNSLRLSCAASGFTFSSFGMSWVRQAPGKGLEWVSSISGSGSDTLYADSVKGRFTISRDNAKTTLYLQMNSLRPEDTALYYCTIGGSLSRSSQGTLVTVSSAA

SEQ ID NO: 120 - protein, 118 aa, Artificial Sequence
  Nanobody Sequence
EVQLVESGGGVVQPGNSLRLSCAASGFTFSSFGMSWVRQAPGKGLEWVSSISGSGSDTLYADSVKGRFTISRDNAKTTLYLQMNSLRPEDTALYYCTIGGSLSRSSQGTLVTVSSAAA

SEQ ID NO: 121 - protein, 116 aa, Artificial Sequence
  Nanobody Sequence
EVQLVESGGGVVQPGNSLRLSCAASGFTFSSFGMSWVRQAPGKGLEWVSSISGSGSDTLYADSVKGRFTISRDNAKTTLYLQMNSLRPEDTALYYCTIGGSLSRSSQGTLVTVSSG

SEQ ID NO: 122 - protein, 117 aa, Artificial Sequence
  Nanobody Sequence
EVQLVESGGGVVQPGNSLRLSCAASGFTFSSFGMSWVRQAPGKGLEWVSSISGSGSDTLYADSVKGRFTISRDNAKTTLYLQMNSLRPEDTALYYCTIGGSLSRSSQGTLVTVSSGG

SEQ ID NO: 123 - protein, 118 aa, Artificial Sequence
  Nanobody Sequence
EVQLVESGGGVVQPGNSLRLSCAASGFTFSSFGMSWVRQAPGKGLEWVSSISGSGSDTLYADSVKGRFTISRDNAKTTLYLQMNSLRPEDTALYYCTIGGSLSRSSQGTLVTVSSGGG

SEQ ID NO: 124 - protein, 5 aa, Artificial Sequence
  CDR 1
SFGMS

SEQ ID NO: 125 - protein, 17 aa, Artificial Sequence
  CDR 2
SISGSGSDTLYADSVKG

SEQ ID NO: 126 - protein, 6 aa, Artificial Sequence
  CDR 3
GGSLSR

SEQ ID NO: 127 - protein, 5 aa, Artificial Sequence
  Linker
GGGGS

SEQ ID NO: 128 - protein, 7 aa, Artificial Sequence
  Linker
SGGSGGS

SEQ ID NO: 129 - protein, 9 aa, Artificial Sequence
  Linker
GGGGSGGGS

SEQ ID NO: 130 - protein, 10 aa, Artificial Sequence
  Linker
GGGGSGGGGS

SEQ ID NO: 131 - protein, 15 aa, Artificial Sequence
  Linker
GGGGSGGGGSGGGGS

SEQ ID NO: 132 - protein, 18 aa, Artificial Sequence
  Linker
GGGGSGGGGSGGGGGGGS

SEQ ID NO: 133 - protein, 20 aa, Artificial Sequence
  Linker
GGGGSGGGGSGGGGSGGGGS

SEQ ID NO: 134 - protein, 25 aa, Artificial Sequence
  Linker
GGGGSGGGGSGGGGSGGGGSGGGGS

SEQ ID NO: 135 - protein, 30 aa, Artificial Sequence
  Linker
GGGGSGGGGSGGGGSGGGGSGGGGSGGGGS

SEQ ID NO: 136 - protein, 35 aa, Artificial Sequence
  Linker
GGGGSGGGGSGGGGSGGGGSGGGGSGGGGSGGGGS